European Patent Specification EP 3 354 723 B1, published December 13, 2023. Title: MEDIA FOR CULTURING STEM CELLS. Applicant: Technion Research and Development of Foundation, Ltd. Application 06766237.9. The sequence listing filed with the application follows.

SEQUENCE LISTING (31 sequences)

SEQ ID NO: 1 - DNA, 23 bp, Artificial sequence
  Single strand DNA oligonucleotide
gagaacaatgagaaccttcagga

SEQ ID NO: 2 - DNA, 23 bp, Artificial sequence
  Single strand DNA oligonucleotide
ttctggcgccggttacagaacca

SEQ ID NO: 3 - DNA, 24 bp, Artificial sequence
  Single strand DNA oligonucleotide
tgcttgaatgtgctgatgacaggg

SEQ ID NO: 4 - DNA, 24 bp, Artificial sequence
  Single strand DNA oligonucleotide
aaggcaagtcagcagccatctcat

SEQ ID NO: 5 - DNA, 25 bp, Artificial sequence
  Single strand DNA oligonucleotide
gctggattgtctgcaggatggggaa

SEQ ID NO: 6 - DNA, 25 bp, Artificial sequence
  Single strand DNA oligonucleotide
tcccctgaagaaaattggttaaaat

SEQ ID NO: 7 - DNA, 22 bp, Artificial sequence
  Single strand DNA oligonucleotide
gagtgaaatggcacgataccta

SEQ ID NO: 8 - DNA, 22 bp, Artificial sequence
  Single strand DNA oligonucleotide
tttcctctccttcttcaccttc

SEQ ID NO: 9 - DNA, 22 bp, Artificial sequence
  Single strand DNA oligonucleotide
ggagttatggtgggtatgggtc

SEQ ID NO: 10 - DNA, 22 bp, Artificial sequence
  Single strand DNA oligonucleotide
agtggtgacaaaggagtagcca

SEQ ID NO: 11 - DNA, 32 bp, Artificial sequence
  Single strand DNA oligonucleotide
atctggcaccacaccttctacaatgagctgcg

SEQ ID NO: 12 - DNA, 32 bp, Artificial sequence
  Single strand DNA oligonucleotide
cgtcatactcctgcttgctgatccacatctgc

SEQ ID NO: 13 - DNA, 18 bp, Artificial sequence
  Single strand DNA oligonucleotide
cccccggcggcaatagca

SEQ ID NO: 14 - DNA, 20 bp, Artificial sequence
  Single strand DNA oligonucleotide
tcggcgccggggagatacat

SEQ ID NO: 15 - DNA, 23 bp, Artificial sequence
  Single strand DNA oligonucleotide
gcgtacgcaaattaaagtccaga

SEQ ID NO: 16 - DNA, 25 bp, Artificial sequence
  Single strand DNA oligonucleotide
cagcatcctaaacagctcgcagaat

SEQ ID NO: 17 - DNA, 23 bp, Artificial sequence
  Single strand DNA oligonucleotide
taccatgcgaccagtggtgcgct

SEQ ID NO: 18 - DNA, 23 bp, Artificial sequence
  Single strand DNA oligonucleotide
gaattctggttatcatcggggaa

SEQ ID NO: 19 - DNA, 23 bp, Artificial sequence
  Single strand DNA oligonucleotide
ctacaacgcctacgagtcctaca

SEQ ID NO: 20 - DNA, 24 bp, Artificial sequence
  Single strand DNA oligonucleotide
gttgcaccagaaaagtcagagttg

SEQ ID NO: 21 - DNA, 25 bp, Artificial sequence
  Single strand DNA oligonucleotide
ctcagtgatcctgatcagatgaacg

SEQ ID NO: 22 - DNA, 25 bp, Artificial sequence
  Single strand DNA oligonucleotide
agtccctggcggcaagattatcaag

SEQ ID NO: 23 - DNA, 25 bp, Artificial sequence
  Single strand DNA oligonucleotide
acctgactcctgaggagaagtctgc

SEQ ID NO: 24 - DNA, 25 bp, Artificial sequence
  Single strand DNA oligonucleotide
tagccacaccagccaccactttctg

SEQ ID NO: 25 - DNA, 20 bp, Artificial sequence
  Single strand DNA oligonucleotide
atgcacggcatctgggaatc

SEQ ID NO: 26 - DNA, 24 bp, Artificial sequence
  Single strand DNA oligonucleotide
gctactgtcctgcaagttgctgtc

SEQ ID NO: 27 - DNA, 20 bp, Artificial sequence
  Single strand DNA oligonucleotide
cagtctgaccagcgtgaaaa

SEQ ID NO: 28 - DNA, 20 bp, Artificial sequence
  Single strand DNA oligonucleotide
ggccatccaaatctgtccta

SEQ ID NO: 29 - DNA, 20 bp, Artificial sequence
  Single strand DNA oligonucleotide
actaacatgagtgtggatcc

SEQ ID NO: 30 - DNA, 20 bp, Artificial sequence
  Single strand DNA oligonucleotide
tcatcttcacacgtcttcag

SEQ ID NO: 31 - protein, 543 aa, Artificial sequence
  IL6R/IL6 chimeric protein
MLAVGCALLAALLAAPGAALAPRRCPAQEVARGVLTSLPGDSVTLTCPGVEPEDNATVHWVLRKPAAGSHPSRWAGMGRRLLLRSVQLHDSGNYSCYRAGRPAGTVHLLVDVPPEEPQLSCFRKSPLSNVVCEWGPRSTPSLTTKAVLLVRKFQNSPAEDFQEPCQYSQESQKFSCQLAVPEGDSSFYIVSMCVASSVGSKFSKTQTFQGCGILQPDPPANITVTAVARNPRWLSVTWQDPHSWNSSFYRLRFELRYRAERSKTFTTWMVKDLQHHCVIHDAWSGLRHVVQLRAQEEFGQGEWSEWSPEAMGTPWTESRSPPAENEVSTPMQALTTNKDDDNILFRDSANATSLPVEFMPVPPGEDSKDVAAPHRQPLTSSERIDKQIRYILDGISALRKETCNKSNMCESSKEALAENNLNLPKMAEKDGCFQSGFNEETCLVKIITGLLEFEVYLEYLQNRFESSEEQARAVQMSTKVLIQFLQKKAKNLDAITTPDPTTNASLLTKLQAQNQWLQDMTTHLILRSFKEFLQSSLRALRQM